European Patent Application EP 4 230 638 A1, published August 23, 2023. Title: Peptides and compositions for use in cosmetics. Applicant: Lipotrue S.L. The sequence listing filed with the application follows.

SEQUENCE LISTING (7 sequences)

SEQ ID NO: 1 - protein, 6 aa, Takifugu rubripes
  Peptide derived from the sequence of Nucleolar complex protein 2 homolog of the puffer fish Takifugu rubripes (Uniprot reference number: H2TGB2, amino acids 88 to 93).
RWQKNQ

SEQ ID NO: 2 - protein, 6 aa, Takifugu rubripes
  Peptide derived from the sequence of Disabled homolog 2-interacting protein-like isoform X2 (Synaptic Ras-GTPase activating domain) (NCBI Reference Sequence: XP_003976523.1, amino acids 64 to 68).
KRRYYC

SEQ ID NO: 3 - protein, 5 aa, Takifugu rubripes
  Peptide derived from a genome sequence predicted as calcium-independent phospholipase A2-gamma-like isoform X2 (NCBI Reference Sequence: XP_011605802.2, amino acids 7 to 11)
KHRSY

SEQ ID NO: 4 - protein, 5 aa, Artificial Sequence
  Artificially synthesized sequence
KDRVY

SEQ ID NO: 5 - protein, 6 aa, Artificial Sequence
  Artificially synthesized sequence
IEPYYV

SEQ ID NO: 6 - protein, 6 aa, Artificial Sequence
  Artificially synthesized sequence
KKHFWA

SEQ ID NO: 7 - protein, 6 aa, Artificial Sequence
  Artificially synthesized sequence
  VARIANT 1: Xaa is selected from Lys, Arg or His
  VARIANT 2: Xaa is selected from Lys, Arg, His, Asp or Glu
  VARIANT 3: Xaa is selected from Lys, Arg or His
  VARIANT 4: Xaa is selected from Gly, Ala, Val, Leu, Met, Ile, Ser, Thr, Cys, Pro, Asn, Gln, Phe, Tyr or Trp
  VARIANT 5: Xaa is selected from Phe, Tyr or Trp
  VARIANT 6: Xaa is absent or is selected from Gly, Ala, Val, Leu, Met, Ile, Ser, Thr, Cys, Pro, Asn or Gln
XXXXXX